European Patent Specification EP 3 362 475 B1, published August 30, 2023. Title: CD73 BLOCKING AGENTS. Applicant: INNATE PHARMA CENTRE LEON BERARD. The sequence listing filed with the application follows.

SEQUENCE LISTING (107 sequences)

SEQ ID NO: 1 - protein, 574 aa, homo sapiens
MCPRAARAPATLLLALGAVLWPAAGAWELTILHTNDVHSRLEQTSEDSSKCVNASRCMGGVARLFTKVQQIRRAEPNVLLLDAGDQYQGTIWFTVYKGAEVAHFMNALRYDAMALGNHEFDNGVEGLIEPLLKEAKFPILSANIKAKGPLASQISGLYLPYKVLPVGDEVVGIVGYTSKETPFLSNPGTNLVFEDEITALQPEVDKLKTLNVNKIIALGHSGFEMDKLIAQKVRGVDVVVGGHSNTFLYTGNPPSKEVPAGKYPFIVTSDDGRKVPVVQAYAFGKYLGYLKIEFDERGNVISSHGNPILLNSSIPEDPSIKADINKWRIKLDNYSTQELGKTIVYLDGSSQSCRFRECNMGNLICDAMINNNLRHTDEMFWNHVSMCILNGGGIRSPIDERNNGTITWENLAAVLPFGGTFDLVQLKGSTLKKAFEHSVHRYGQSTGEFLQVGGIHVVYDLSRKPGDRVVKLDVLCTKCRVPSYDPLKMDEVYKVILPNFLANGGDGFQMIKDELLRHDSGDQDINVVSTYISKMKVIYPAVEGRIKFSTGSHCHGSFSLIFLSLWAVIFVLYQ

SEQ ID NO: 2 - protein, 553 aa, homo sapiens
MCPRAARAPATLLLALGAVLWPAAGAWELTILHTNDVHSRLEQTSEDSSKCVNASRCMGGVARLFTKVQQIRRAEPNVLLLDAGDQYQGTIWFTVYKGAEVAHFMNALRYDAMALGNHEFDNGVEGLIEPLLKEAKFPILSANIKAKGPLASQISGLYLPYKVLPVGDEVVGIVGYTSKETPFLSNPGTNLVFEDEITALQPEVDKLKTLNVNKIIALGHSGFEMDKLIAQKVRGVDVVVGGHSNTFLYTGNPPSKEVPAGKYPFIVTSDDGRKVPVVQAYAFGKYLGYLKIEFDERGNVISSHGNPILLNSSIPEDPSIKADINKWRIKLDNYSTQELGKTIVYLDGSSQSCRFRECNMGNLICDAMINNNLRHTDEMFWNHVSMCILNGGGIRSPIDERNNGTITWENLAAVLPFGGTFDLVQLKGSTLKKAFEHSVHRYGQSTGEFLQVGGIHVVYDLSRKPGDRVVKLDVLCTKCRVPSYDPLKMDEVYKVILPNFLANGGDGFQMIKDELLRHDSGDQDINVVSTYISKMKVIYPAVEGRIKHHHHHH

SEQ ID NO: 3 - protein, 117 aa, mus musculus
DVQLQESGPGLVKPSQSLSLTCTVTGYSITSDYAWNWIRQFPGNKLEWMGYIIYSGSTSYNPSLNSRISITRDTSKNQFFLQLNSVTTEDTATYYCAREAYLYFDYWGQGTTLTVSS

SEQ ID NO: 4 - protein, 107 aa, mus musculus
DIQMTQTTSSLSASLGDRVTISCRASQDINNYLNWYQQKPDGTVKLLIYYTSRLHSGVPSRFSGSGSGTDYSLTISNLEREDVATYFCQQGNTLPWTFGGGTKLEIK

SEQ ID NO: 5 - protein, 6 aa, mus musculus
SDYAWN

SEQ ID NO: 6 - protein, 8 aa, mus musculus
GYSITSDY

SEQ ID NO: 7 - protein, 9 aa, mus musculus
GYSITSDYA

SEQ ID NO: 8 - protein, 16 aa, mus musculus
YIIYSGSTSYNPSLNS

SEQ ID NO: 9 - protein, 3 aa, mus musculus
YSG

SEQ ID NO: 10 - protein, 7 aa, mus musculus
IIYSGST

SEQ ID NO: 11 - protein, 8 aa, mus musculus
EAYLYFDY

SEQ ID NO: 12 - protein, 6 aa, mus musculus
AYLYFD

SEQ ID NO: 13 - protein, 10 aa, mus musculus
AREAYLYFDY

SEQ ID NO: 14 - protein, 11 aa, mus musculus
RASQDINNYLN

SEQ ID NO: 15 - protein, 7 aa, mus musculus
SQDINNY

SEQ ID NO: 16 - protein, 6 aa, mus musculus
QDINNY

SEQ ID NO: 17 - protein, 7 aa, mus musculus
YTSRLHS

SEQ ID NO: 18 - protein, 3 aa, mus musculus
YTS

SEQ ID NO: 19 - protein, 9 aa, mus musculus
QQGNTLPWT

SEQ ID NO: 20 - protein, 6 aa, mus musculus
GNTLPW

SEQ ID NO: 21 - protein, 120 aa, mus musculus
QVQLQQSGPELVKPGASVRISCKASGYTFTNYYIHWVKQRPGQGLEWIGWIYPGNVNTKYNEKFKGKATLTADKSSNTAYMQLSSLTSEDSAVYFCAREGGYDRYALDYWGQGTSVTVSS

SEQ ID NO: 22 - protein, 106 aa, mus musculus
QIVLTQSPALMSASPGEKVTMTCSASSSVSYMYWYQQKPRSSPKPWIYLTSNLASGVPARFSGSGSGTSYSLTISSMEAEDAATYYCQQWSSNPLTFGAGTKLELK

SEQ ID NO: 23 - protein, 5 aa, mus musculus
NYYIH

SEQ ID NO: 24 - protein, 7 aa, mus musculus
GYTFTNY

SEQ ID NO: 25 - protein, 8 aa, mus musculus
GYTFTNYY

SEQ ID NO: 26 - protein, 17 aa, mus musculus
WIYPGNVNTKYNEKFKG

SEQ ID NO: 27 - protein, 4 aa, mus musculus
PGNV

SEQ ID NO: 28 - protein, 8 aa, mus musculus
IYPGNVNT

SEQ ID NO: 29 - protein, 11 aa, mus musculus
EGGYDRYALDY

SEQ ID NO: 30 - protein, 9 aa, mus musculus
GGYDRYALD

SEQ ID NO: 31 - protein, 13 aa, mus musculus
AREGGYDRYALDY

SEQ ID NO: 32 - protein, 10 aa, mus musculus
SASSSVSYMY

SEQ ID NO: 33 - protein, 6 aa, mus musculus
SSSVSY

SEQ ID NO: 34 - protein, 5 aa, mus musculus
SSVSY

SEQ ID NO: 35 - protein, 7 aa, mus musculus
LTSNLAS

SEQ ID NO: 36 - protein, 3 aa, mus musculus
LTS

SEQ ID NO: 37 - protein, 9 aa, mus musculus
QQWSSNPLT

SEQ ID NO: 38 - protein, 9 aa, mus musculus
LTSWSSNPL

SEQ ID NO: 39 - protein, 9 aa, mus musculus
QQWSSNPLT

SEQ ID NO: 40 - protein, 119 aa, mus musculus
QVQLQQPGAEVVKPGASVKLSCKASGYTFTSYWMHWVKQRPGQGLEWIGEINPSNGRTNYNEKFKSKATLTVDKSSSTAYMQLSNLTSEDSAVYYCARRGGYGNWFAYWGQGTLVTVSA

SEQ ID NO: 41 - protein, 107 aa, mus musculus
DIKMTQSPSSMYASLGERVTITCKASQDINTYLSWFQQKPGKSPKTLIYRANRLVDGVPSRFSGSGSGQDYSLTISSLEYEDMGIYYCLQYDEFPYTFGGGTKLEIK

SEQ ID NO: 42 - protein, 120 aa, mus musculus; identical to SEQ ID NO: 21

SEQ ID NO: 43 - protein, 106 aa, mus musculus; identical to SEQ ID NO: 22

SEQ ID NO: 44 - protein, 122 aa, mus musculus
EVQLQQSGPELVKPGASVKMSCKASGYTFTSYVMHWVKQKPGQGLEWIGYINPYNDGTKYNEKFKGKATLTSDKSSSTAYMELSSLTSEDSAVYYCARWGYDEGYYYAMDYWGQGTSVTVSS

SEQ ID NO: 45 - protein, 107 aa, mus musculus
DIVMTQSPSSMYASLGERVTITCKASQDINSYLSWFQQKPGKSPKTLIYRANRLVDGVPSRFSGSGSGQDYSLTISSLEYEDMGIYYCLQYDEFPLTFGAGTKLELK

SEQ ID NO: 46 - protein, 118 aa, mus musculus
QIQLQQSGAELVKPGASVNLSCKTSGFTFSSSYISWLKQKPGQSLEWIAWIYAGTGTTRYNQKFTGKAQLTVDTSSRTAYMQFSSLTTEDSAIYYCARHVNWDHFEYWGQGTTLTVSS

SEQ ID NO: 47 - protein, 107 aa, mus musculus
DIVMTQSHKFMATSVGDRVNITCKASQDVSTAVAWYQQKPGQSPKLLLYWASTRQTGVPDHFTGSGSGTDYTLTINSVQADDLALYYCQQYYRTPWTFGGGTKLEIK

SEQ ID NO: 48 - protein, 5 aa, mus musculus
SYWMH

SEQ ID NO: 49 - protein, 7 aa, mus musculus
GYTFTSY

SEQ ID NO: 50 - protein, 8 aa, mus musculus
GYTFTSYW

SEQ ID NO: 51 - protein, 17 aa, mus musculus
EINPSNGRTNYNEKFKS

SEQ ID NO: 52 - protein, 10 aa, mus musculus
RGGYGNWFAY

SEQ ID NO: 53 - protein, 8 aa, mus musculus
GGYGNWFA

SEQ ID NO: 54 - protein, 12 aa, mus musculus
ARRGGYGNWFAY

SEQ ID NO: 55 - protein, 5 aa, mus musculus
SYVMH

SEQ ID NO: 56 - protein, 4 aa, mus musculus
PSNG

SEQ ID NO: 57 - protein, 8 aa, mus musculus
GYTFTSYV

SEQ ID NO: 58 - protein, 17 aa, mus musculus
YINPYNDGTKYNEKFKG

SEQ ID NO: 59 - protein, 4 aa, mus musculus
PYND

SEQ ID NO: 60 - protein, 8 aa, mus musculus
INPYNDGT

SEQ ID NO: 61 - protein, 13 aa, mus musculus
WGYDEGYYYAMDY

SEQ ID NO: 62 - protein, 11 aa, mus musculus
GYDEGYYYAMD

SEQ ID NO: 63 - protein, 15 aa, mus musculus
ARWGYDEGYYYAMDY

SEQ ID NO: 64 - protein, 5 aa, mus musculus
SSYIS

SEQ ID NO: 65 - protein, 7 aa, mus musculus
GFTFSSS

SEQ ID NO: 66 - protein, 8 aa, mus musculus
GFTFSSSY

SEQ ID NO: 67 - protein, 17 aa, mus musculus
WIYAGTGTTRYNQKFTG

SEQ ID NO: 68 - protein, 4 aa, mus musculus
AGTG

SEQ ID NO: 69 - protein, 8 aa, mus musculus
IYAGTGTT

SEQ ID NO: 70 - protein, 9 aa, mus musculus
HVNWDHFEY

SEQ ID NO: 71 - protein, 7 aa, mus musculus
VNWDHFE

SEQ ID NO: 72 - protein, 11 aa, mus musculus
ARHVNWDHFEY

SEQ ID NO: 73 - protein, 11 aa, mus musculus
KASQDINTYLS

SEQ ID NO: 74 - protein, 7 aa, mus musculus
SQDINTY

SEQ ID NO: 75 - protein, 6 aa, mus musculus
QDINTY

SEQ ID NO: 76 - protein, 7 aa, mus musculus
RANRLVD

SEQ ID NO: 77 - protein, 3 aa, mus musculus
RAN

SEQ ID NO: 78 - protein, 9 aa, mus musculus
LQYDEFPYT

SEQ ID NO: 79 - protein, 6 aa, mus musculus
YDEFPY

SEQ ID NO: 80 - protein, 11 aa, mus musculus
KASQDINSYLS

SEQ ID NO: 81 - protein, 7 aa, mus musculus
SQDINSY

SEQ ID NO: 82 - protein, 6 aa, mus musculus
QDINSY

SEQ ID NO: 83 - protein, 9 aa, mus musculus
LQYDEFPLT

SEQ ID NO: 84 - protein, 6 aa, mus musculus
YDEFPL

SEQ ID NO: 85 - protein, 11 aa, mus musculus
KASQDVSTAVA

SEQ ID NO: 86 - protein, 7 aa, mus musculus
SQDVSTA

SEQ ID NO: 87 - protein, 6 aa, mus musculus
QDVSTA

SEQ ID NO: 88 - protein, 7 aa, mus musculus
WASTRQT

SEQ ID NO: 89 - protein, 3 aa, mus musculus
WAS

SEQ ID NO: 90 - protein, 9 aa, mus musculus
QQYYRTPWT

SEQ ID NO: 91 - protein, 6 aa, mus musculus
YYRTPW

SEQ ID NO: 92 - protein, 8 aa, mus musculus
INPSNGRT

SEQ ID NO: 93 - protein, 5 aa, Mus musculus
SYNMY

SEQ ID NO: 94 - DNA, 5 bp, Mus musculus
  misc_feature (3)..(3): n is a, c, g, or t
  misc_feature (5)..(5): n is a, c, g, or t
synmn

SEQ ID NO: 95 - protein, 17 aa, Mus musculus
YIDPYNGGTSYNQKFKG

SEQ ID NO: 96 - protein, 17 aa, Mus musculus
YIDPYNGGSSYNQKFKG

SEQ ID NO: 97 - protein, 17 aa, Mus musculus
YIDPYNGGSSYNLTFKG

SEQ ID NO: 98 - protein, 11 aa, Mus musculus
GYGNYKAWFAY

SEQ ID NO: 99 - protein, 11 aa, Mus musculus
GYNNYKAWFAY

SEQ ID NO: 100 - protein, 11 aa, Mus musculus
KASQSVTNDVA

SEQ ID NO: 101 - protein, 11 aa, Mus musculus
KASQSVSNDVA

SEQ ID NO: 102 - protein, 7 aa, Mus musculus
YASNRYT

SEQ ID NO: 103 - protein, 8 aa, Mus musculus
QQDYSSLT

SEQ ID NO: 104 - protein, 330 aa, homo sapiens
ASTKGPSVFPLAPSSKSTSGGTAALGCLVKDYFPEPVTVSWNSGALTSGVHTFPAVLQSSGLYSLSSVVTVPSSSLGTQTYICNVNHKPSNTKVDKRVEPKSCDKTHTCPPCPAPEAEGGPSVFLFPPKPKDTLMISRTPEVTCVVVDVSHEDPEVKFNWYVDGVEVHNAKTKPREEQYNSTYRVVSVLTVLHQDWLNGKEYKCKVSNKALPASIEKTISKAKGQPREPQVYTLPPSREEMTKNQVSLTCLVKGFYPSDIAVEWESNGQPENNYKTTPPVLDSDGSFFLYSKLTVDKSRWQQGNVFSCSVMHEALHNHYTQKSLSLSPGK

SEQ ID NO: 105 - protein, 330 aa, homo sapiens
ASTKGPSVFPLAPSSKSTSGGTAALGCLVKDYFPEPVTVSWNSGALTSGVHTFPAVLQSSGLYSLSSVVTVPSSSLGTQTYICNVNHKPSNTKVDKRVEPKSCDKTHTCPPCPAPEFEGGPSVFLFPPKPKDTLMISRTPEVTCVVVDVSHEDPEVKFNWYVDGVEVHNAKTKPREEQYNSTYRVVSVLTVLHQDWLNGKEYKCKVSNKALPASIEKTISKAKGQPREPQVYTLPPSREEMTKNQVSLTCLVKGFYPSDIAVEWESNGQPENNYKTTPPVLDSDGSFFLYSKLTVDKSRWQQGNVFSCSVMHEALHNHYTQKSLSLSPGK

SEQ ID NO: 106 - protein, 330 aa, homo sapiens
ASTKGPSVFPLAPSSKSTSGGTAALGCLVKDYFPEPVTVSWNSGALTSGVHTFPAVLQSSGLYSLSSVVTVPSSSLGTQTYICNVNHKPSNTKVDKRVEPKSCDKTHTCPPCPAPEAEGAPSVFLFPPKPKDTLMISRTPEVTCVVVDVSHEDPEVKFNWYVDGVEVHNAKTKPREEQYNSTYRVVSVLTVLHQDWLNGKEYKCKVSNKALPSSIEKTISKAKGQPREPQVYTLPPSREEMTKNQVSLTCLVKGFYPSDIAVEWESNGQPENNYKTTPPVLDSDGSFFLYSKLTVDKSRWQQGNVFSCSVMHEALHNHYTQKSLSLSPGK

SEQ ID NO: 107 - protein, 330 aa, Homo sapiens
ASTKGPSVFPLAPSSKSTSGGTAALGCLVKDYFPEPVTVSWNSGALTSGVHTFPAVLQSSGLYSLSSVVTVPSSSLGTQTYICNVNHKPSNTKVDKRVEPKSCDKTHTCPPCPAPEAEGAPSVFLFPPKPKDTLMISRTPEVTCVVVDVSHEDPEVKFNWYVDGVEVHNAKTKPREEQYNSTYRVVSVLTVLHQDWLNGKEYKCKVSNKALPASIEKTISKAKGQPREPQVYTLPPSREEMTKNQVSLTCLVKGFYPSDIAVEWESNGQPENNYKTTPPVLDSDGSFFLYSKLTVDKSRWQQGNVFSCSVMHEALHNHYTQKSLSLSPGK